European Patent Application EP 4 803 547 A1, published September 9, 2026. Title: ANTI-PD-1/CD40 BISPECIFIC ANTIBODY AND USE THEREOF. Applicant: BIONTECH (ZHUHAI) PHARMACEUTICALS R&D CO., LTD. Application CN PCT/CN2024/129694, filed November 4, 2024. The sequence listing filed with the application follows.

SEQUENCE LISTING (49 sequences)

SEQ ID NO: 1 - protein, 709 aa, synthetic construct
  source 1..709: note = PD-1xCD40 (ADI55164)-HC
QVQLVQSGAEVKKPGASVKVSCKASGYTFTEYYIYWVRQAPGQGLEWIGGINPSNGGTNFNEKFKPRVTMTVDTSTSTAYMELSSLRSEDTAVYYCTVRDFRFDKGFKYWGQGTLVTVSSASTKGPSVFPLAPSSKSTSGGTAALGCLVKDYFPEPVTVSWNSGALTSGVHTFPAVLQSSGLYSLSSVVTVPSSSLGTQTYICNVNHKPSNTKVDKKVEPKSCDKTHTCPPCPAPEAAGAPSVFLFPPKPKDTLMISRTPEVTCVVVDVSHEDPEVKFNWYVDGVEVHNAKTKPREEQYNSTYRVVSVLTVLHQDWLNGKEYKCKVSNKALPAPIEKTISKAKGQPREPQVYTLPPSRDELTKNQVSLTCLVKGFYPSDIAVEWESNGQPENNYKTTPPVLDSDGSFFLYSKLTVDKSRWQQGNVFSCSVMHEALHNHYTQKSLSLSPGGGGGAGGGGAEVQLVESGGGLVQPGRSLRLSCAASGFTFDDYAMHWVRQAPGKCLEWVSGISWSSDSIHYADSVKGRFTISRDNAKNSLYLQMNSLRAEDTAVYYCAKDPTATTGARGYFDLWGRGTLVTVSSGGGGSGGGGSGGGGSGGGGSDIQMTQSPSSVSASVGDRVTITCRASKVISSWLAWYQQKPGKAPKLLIYAASYLESGVPSRFSGSGSGTDFTLTISSLQPEDFATYYCQQHSSFPPTFGCGTKVEIK

SEQ ID NO: 2 - protein, 705 aa, synthetic construct
  source 1..705: note = PD-1xCD40 (ADI55147)-HC
QVQLVQSGAEVKKPGASVKVSCKASGYTFTEYYIYWVRQAPGQGLEWIGGINPSNGGTNFNEKFKPRVTMTVDTSTSTAYMELSSLRSEDTAVYYCTVRDFRFDKGFKYWGQGTLVTVSSASTKGPSVFPLAPSSKSTSGGTAALGCLVKDYFPEPVTVSWNSGALTSGVHTFPAVLQSSGLYSLSSVVTVPSSSLGTQTYICNVNHKPSNTKVDKKVEPKSCDKTHTCPPCPAPEAAGAPSVFLFPPKPKDTLMISRTPEVTCVVVDVSHEDPEVKFNWYVDGVEVHNAKTKPREEQYNSTYRVVSVLTVLHQDWLNGKEYKCKVSNKALPAPIEKTISKAKGQPREPQVYTLPPSRDELTKNQVSLTCLVKGFYPSDIAVEWESNGQPENNYKTTPPVLDSDGSFFLYSKLTVDKSRWQQGNVFSCSVMHEALHNHYTQKSLSLSPGGGGGAGGGGAQVQLVESGGGVVQPGRSLRLSCAASGFTFGSYGMHWVRQAPGKCLEWVAVISYEGVKKYYADSVKGRFTISRDNSKNTLYLQMNSLRAEDTAVYYCARDTSRGHDIWGQGTMVTVSSGGGGSGGGGSGGGGSGGGGSEIVLTQSPGTLSLSPGERATLSCRASQSVSYDYLAWYQQKPGQAPRLLIYGASARANGIPDRFSGSGSGTDFTLTISRLEPEDFAVYYCQQYADYPPFTFGCGTKVEIK

SEQ ID NO: 3 - protein, 120 aa, synthetic construct
  source 1..120: note = Anti-PD1 (ADI-54872) VH; note (original language) = Anti-PD1（ADI-54872） VH
QVQLVQSGAEVKKPGASVKVSCKASGYTFTEYYIYWVRQAPGQGLEWIGGINPSNGGTNFNEKFKPRVTMTVDTSTSTAYMELSSLRSEDTAVYYCTVRDFRFDKGFKYWGQGTLVTVSS

SEQ ID NO: 4 - protein, 111 aa, synthetic construct
  source 1..111: note = Anti-PD1 (ADI-54872) VL; note (original language) = Anti-PD1（ADI-54872） VL
EIVLTQSPATLSLSPGERATLSCRASKSVSTSGLNYVHWYQRKPGQAPRLLIYLGSYLDSGVPARFSGSGSGTDFTLTISSLEPEDFAVYYCQQSWELPLTFGGGTKVEIK

SEQ ID NO: 5 - protein, 123 aa, synthetic construct
  source 1..123: note = ADI-55164 VH (anti CD40)
EVQLVESGGGLVQPGRSLRLSCAASGFTFDDYAMHWVRQAPGKGLEWVSGISWSSDSIHYADSVKGRFTISRDNAKNSLYLQMNSLRAEDTAVYYCAKDPTATTGARGYFDLWGRGTLVTVSS

SEQ ID NO: 6 - protein, 117 aa, synthetic construct
  source 1..117: note = ADI-55147 VH (anti CD40)
QVQLVESGGGVVQPGRSLRLSCAASGFTFGSYGMHWVRQAPGKGLEWVAVISYEGVKKYYADSVKGRFTISRDNSKNTLYLQMNSLRAEDTAVYYCARDTSRGHDIWGQGTMVTVSS

SEQ ID NO: 7 - protein, 8 aa, synthetic construct
  source 1..8: note = ADI-55164 HCDR1 (IMGT); note (original language) = ADI-55164 HCDR1（IMGT）
GFTFDDYA

SEQ ID NO: 8 - protein, 8 aa, synthetic construct
  source 1..8: note = ADI-55164 HCDR2 (IMGT); note (original language) = ADI-55164 HCDR2（IMGT）
ISWSSDSI

SEQ ID NO: 9 - protein, 16 aa, synthetic construct
  source 1..16: note = ADI-55164 HCDR3 (IMGT); note (original language) = ADI-55164 HCDR3（IMGT）
AKDPTATTGARGYFDL

SEQ ID NO: 10 - protein, 8 aa, synthetic construct
  source 1..8: note = ADI-55147 HCDR1 (IMGT); note (original language) = ADI-55147 HCDR1（IMGT）
GFTFGSYG

SEQ ID NO: 11 - protein, 8 aa, synthetic construct
  source 1..8: note = ADI-55147 HCDR2 (IMGT); note (original language) = ADI-55147 HCDR2（IMGT）
ISYEGVKK

SEQ ID NO: 12 - protein, 10 aa, synthetic construct
  source 1..10: note = ADI-55147 HCDR3 (IMGT); note (original language) = ADI-55147 HCDR3（IMGT）
ARDTSRGHDI

SEQ ID NO: 13 - protein, 8 aa, synthetic construct
  source 1..8: note = Anti-PD1 (ADI-54872) HCDR1 (IMGT); note (original language) = Anti-PD1 (ADI-54872) HCDR1（IMGT）
GYTFTEYY

SEQ ID NO: 14 - protein, 8 aa, synthetic construct
  source 1..8: note = Anti-PD1 (ADI-54872) HCDR2 (IMGT); note (original language) = Anti-PD1 (ADI-54872) HCDR2（IMGT）
INPSNGGT

SEQ ID NO: 15 - protein, 13 aa, synthetic construct
  source 1..13: note = Anti-PD1 (ADI-54872) HCDR3 (IMGT); note (original language) = Anti-PD1 (ADI-54872) HCDR3（IMGT）
TVRDFRFDKGFKY

SEQ ID NO: 16 - protein, 10 aa, synthetic construct
  source 1..10: note = Anti-PD1 (ADI-54872) LCDR1 (IMGT); note (original language) = Anti-PD1 (ADI-54872) LCDR1（IMGT）
KSVSTSGLNY

SEQ ID NO: 17 - skipped

SEQ ID NO: 18 - protein, 9 aa, synthetic construct
  source 1..9: note = Anti-PD1 (ADI-54872) LCDR3 (IMGT); note (original language) = Anti-PD1 (ADI-54872) LCDR3（IMGT）
QQSWELPLT

SEQ ID NO: 19 - protein, 329 aa, synthetic construct
  source 1..329: note = Heavy chain constant region; note (original language) = 重链恒定区
ASTKGPSVFPLAPSSKSTSGGTAALGCLVKDYFPEPVTVSWNSGALTSGVHTFPAVLQSSGLYSLSSVVTVPSSSLGTQTYICNVNHKPSNTKVDKKVEPKSCDKTHTCPPCPAPEAAGAPSVFLFPPKPKDTLMISRTPEVTCVVVDVSHEDPEVKFNWYVDGVEVHNAKTKPREEQYNSTYRVVSVLTVLHQDWLNGKEYKCKVSNKALPAPIEKTISKAKGQPREPQVYTLPPSRDELTKNQVSLTCLVKGFYPSDIAVEWESNGQPENNYKTTPPVLDSDGSFFLYSKLTVDKSRWQQGNVFSCSVMHEALHNHYTQKSLSLSPG

SEQ ID NO: 20 - protein, 107 aa, synthetic construct [sequence omitted]

SEQ ID NO: 21 - protein, 126 aa, synthetic construct
  source 1..126: note = CP-870893 VH
QVQLVQSGAEVKKPGASVKVSCKASGYTFTGYYMHWVRQAPGQGLEWMGWINPDSGGTNYAQKFQGRVTMTRDTSISTAYMELNRLRSDDTAVYYCARDQPLGYCTNGVCSYFDYWGQGTLVTVSS

SEQ ID NO: 22 - protein, 107 aa, synthetic construct
  source 1..107: note = CP-870893 VL
DIQMTQSPSSVSASVGDRVTITCRASQGIYSWLAWYQQKPGKAPNLLIYTASTLQSGVPSRFSGSGSGTDFTLTISSLQPEDFATYYCQQANIFPLTFGGGTKVEIK

SEQ ID NO: 23 - protein, 107 aa, synthetic construct
  source 1..107: note = ADI-55164 VL
DIQMTQSPSSVSASVGDRVTITCRASKVISSWLAWYQQKPGKAPKLLIYAASYLESGVPSRFSGSGSGTDFTLTISSLQPEDFATYYCQQHSSFPPTFGGGTKVEIK

SEQ ID NO: 24 - protein, 109 aa, synthetic construct
  source 1..109: note = ADI-55147 VL
EIVLTQSPGTLSLSPGERATLSCRASQSVSYDYLAWYQQKPGQAPRLLIYGASARANGIPDRFSGSGSGTDFTLTISRLEPEDFAVYYCQQYADYPPFTFGGGTKVEIK

SEQ ID NO: 25 - protein, 6 aa, synthetic construct
  source 1..6: note = ADI-55164 LCDR1 (IMGT); note (original language) = ADI-55164 LCDR1（IMGT）
KVISSW

SEQ ID NO: 26 - skipped

SEQ ID NO: 27 - protein, 9 aa, synthetic construct
  source 1..9: note = ADI-55164 LCDR3 (IMGT); note (original language) = ADI-55164 LCDR3（IMGT）
QQHSSFPPT

SEQ ID NO: 28 - protein, 7 aa, synthetic construct
  source 1..7: note = ADI-55147 LCDR1 (IMGT); note (original language) = ADI-55147 LCDR1（IMGT）
QSVSYDY

SEQ ID NO: 29 - skipped

SEQ ID NO: 30 - protein, 10 aa, synthetic construct
  source 1..10: note = ADI-55147 LCDR3 (IMGT); note (original language) = ADI-55147 LCDR3（IMGT）
QQYADYPPFT

SEQ ID NO: 31 - protein, 123 aa, synthetic construct
  source 1..123: note = ADI-55164 VH (G44C substitution mutation); note (original language) = ADI-55164 VH （G44C置换突变）
EVQLVESGGGLVQPGRSLRLSCAASGFTFDDYAMHWVRQAPGKCLEWVSGISWSSDSIHYADSVKGRFTISRDNAKNSLYLQMNSLRAEDTAVYYCAKDPTATTGARGYFDLWGRGTLVTVSS

SEQ ID NO: 32 - protein, 117 aa, synthetic construct
  source 1..117: note = ADI-55147 VH (G44C substitution mutation); note (original language) = ADI-55147 VH （G44C置换突变）
QVQLVESGGGVVQPGRSLRLSCAASGFTFGSYGMHWVRQAPGKCLEWVAVISYEGVKKYYADSVKGRFTISRDNSKNTLYLQMNSLRAEDTAVYYCARDTSRGHDIWGQGTMVTVSS

SEQ ID NO: 33 - protein, 107 aa, synthetic construct
  source 1..107: note = ADI-55164 VL (G100C substitution mutation); note (original language) = ADI-55164 VL (G100C置换突变)
DIQMTQSPSSVSASVGDRVTITCRASKVISSWLAWYQQKPGKAPKLLIYAASYLESGVPSRFSGSGSGTDFTLTISSLQPEDFATYYCQQHSSFPPTFGCGTKVEIK

SEQ ID NO: 34 - protein, 109 aa, synthetic construct
  source 1..109: note = ADI-55147 VL (G102C substitution mutation); note (original language) = ADI-55147 VL （G102C置换突变）
EIVLTQSPGTLSLSPGERATLSCRASQSVSYDYLAWYQQKPGQAPRLLIYGASARANGIPDRFSGSGSGTDFTLTISRLEPEDFAVYYCQQYADYPPFTFGCGTKVEIK

SEQ ID NO: 35 - protein, 218 aa, synthetic construct
  source 1..218: note = LC of bispecific antibody PD-1xCD40
EIVLTQSPATLSLSPGERATLSCRASKSVSTSGLNYVHWYQRKPGQAPRLLIYLGSYLDSGVPARFSGSGSGTDFTLTISSLEPEDFAVYYCQQSWELPLTFGGGTKVEIKRTVAAPSVFIFPPSDEQLKSGTASVVCLLNNFYPREAKVQWKVDNALQSGNSQESVTEQDSKDSTYSLSSTLTLSKADYEKHKVYACEVTHQGLSSPVTKSFNRGEC

SEQ ID NO: 36 - protein, 10 aa, synthetic construct
  source 1..10: note = Linker1
GGGGAGGGGA

SEQ ID NO: 37 - protein, 20 aa, synthetic construct
  source 1..20: note = Linker2
GGGGSGGGGSGGGGSGGGGS

SEQ ID NO: 38 - protein, 709 aa, synthetic construct
  source 1..709: note = PD1(pembro)xCD40 (ADI55164)-HC
EVQLVQSGVEVKKPGASVKVSCKASGYTFTNYYMYWVRQAPGQGLEWMGGINPSNGGTNFNEKFKNRVTLTTDSSTTTAYMELKSLQFDDTAVYYCARRDYRFDMGFDYWGQGTTVTVSSASTKGPSVFPLAPSSKSTSGGTAALGCLVKDYFPEPVTVSWNSGALTSGVHTFPAVLQSSGLYSLSSVVTVPSSSLGTQTYICNVNHKPSNTKVDKKVEPKSCDKTHTCPPCPAPEAAGAPSVFLFPPKPKDTLMISRTPEVTCVVVDVSHEDPEVKFNWYVDGVEVHNAKTKPREEQYNSTYRVVSVLTVLHQDWLNGKEYKCKVSNKALPAPIEKTISKAKGQPREPQVYTLPPSRDELTKNQVSLTCLVKGFYPSDIAVEWESNGQPENNYKTTPPVLDSDGSFFLYSKLTVDKSRWQQGNVFSCSVMHEALHNHYTQKSLSLSPGGGGGAGGGGAEVQLVESGGGLVQPGRSLRLSCAASGFTFDDYAMHWVRQAPGKCLEWVSGISWSSDSIHYADSVKGRFTISRDNAKNSLYLQMNSLRAEDTAVYYCAKDPTATTGARGYFDLWGRGTLVTVSSGGGGSGGGGSGGGGSGGGGSDIQMTQSPSSVSASVGDRVTITCRASKVISSWLAWYQQKPGKAPKLLIYAASYLESGVPSRFSGSGSGTDFTLTISSLQPEDFATYYCQQHSSFPPTFGCGTKVEIK

SEQ ID NO: 39 - protein, 120 aa, synthetic construct
  source 1..120: note = Anti- PD1(pembro) VH
EVQLVQSGVEVKKPGASVKVSCKASGYTFTNYYMYWVRQAPGQGLEWMGGINPSNGGTNFNEKFKNRVTLTTDSSTTTAYMELKSLQFDDTAVYYCARRDYRFDMGFDYWGQGTTVTVSS

SEQ ID NO: 40 - protein, 111 aa, synthetic construct [sequence omitted]

SEQ ID NO: 41 - protein, 8 aa, synthetic construct
  source 1..8: note = Anti- PD1(pembro) HCDR1 (IMGT); note (original language) = Anti- PD1(pembro) HCDR1（IMGT）
GYTFTNYY

SEQ ID NO: 42 - protein, 8 aa, synthetic construct
  source 1..8: note = Anti- PD1(pembro) HCDR2 (IMGT); note (original language) = Anti- PD1(pembro) HCDR2（IMGT）
INPSNGGT

SEQ ID NO: 43 - protein, 13 aa, synthetic construct
  source 1..13: note = Anti- PD1(pembro) HCDR3 (IMGT); note (original language) = Anti- PD1(pembro) HCDR3（IMGT）
ARRDYRFDMGFDY

SEQ ID NO: 44 - protein, 10 aa, synthetic construct
  source 1..10: note = Anti- PD1(pembro) LCDR1 (IMGT); note (original language) = Anti- PD1(pembro) LCDR1（IMGT）
KGVSTSGYSY

SEQ ID NO: 45 - skipped

SEQ ID NO: 46 - protein, 9 aa, synthetic construct
  source 1..9: note = Anti- PD1(pembro) LCDR3 (IMGT); note (original language) = Anti- PD1(pembro) LCDR3（IMGT）
QHSRDLPLT

SEQ ID NO: 47 - protein, 218 aa, synthetic construct
  source 1..218: note = PD1(pembro)xCD40 (ADI55164)-LC
EIVLTQSPATLSLSPGERATLSCRASKGVSTSGYSYLHWYQQKPGQAPRLLIYLASYLESGVPARFSGSGSGTDFTLTISSLEPEDFAVYYCQHSRDLPLTFGGGTKVEIKRTVAAPSVFIFPPSDEQLKSGTASVVCLLNNFYPREAKVQWKVDNALQSGNSQESVTEQDSKDSTYSLSSTLTLSKADYEKHKVYACEVTHQGLSSPVTKSFNRGEC

SEQ ID NO: 48 - protein, 713 aa, synthetic construct
  source 1..713: note = YH008 HC
EVQLVESGGGLVQPGGSLRLSCAASGFTFSSYSMSWVRQAPGKRLEWVAHISSGGSSTYYPDTVKGRFTISRDNSKNTLYLQMNSLRAEDTAMYYCTRQFYYGSSFWYFDVWGAGTTVTVSSASTKGPSVFPLAPSSKSTSGGTAALGCLVKDYFPEPVTVSWNSGALTSGVHTFPAVLQSSGLYSLSSVVTVPSSSLGTQTYICNVNHKPSNTKVDKKVEPKSCDKTHTCPPCPAPEAAGGPSVFLFPPKPKDTLMISRTPEVTCVVVDVSHEDPEVKFNWYVDGVEVHNAKTKPREEQYNSTYRVVSVLTVLHQDWLNGKEYKCKVSNKALPAPIEKTISKAKGQPREPQVYTLPPSREEMTKNQVSLTCLVKGFYPSDIAVEWESNGQPENNYKTTPPVLDSDGSFFLYSKLTVDKSRWQQGNVFSCSVMHEALHNHYTQKSLSLSPGGGGGSGGGGSGGGGSDVVMTQSPLSLPVTLGQPASISCRSSQSLLHSNGNTYLHWYQQRPGQSPNHLIYQVSNRFSGVPDRFSGSGSGTDFTLKISRVEAEDVGVYFCSQTTHVPWTFGCGTKVEIKGGGGSGGGGSGGGGSGGGGSQVQLVQSGAEVKKPGASVKLSCKASGYTFISYYIYWVKQAPGQCLEWIGGINPRNGGTNFNEKFKSRATLTVDTSISTAYMELSRLRSEDTAVYYCTRHGNGVYWGQGTTLTVSS

SEQ ID NO: 49 - protein, 218 aa, synthetic construct
  source 1..218: note = YH008 LC
DNVLTQSPATLSVSPGERATLSCKASQSVDFDGDSYMNWYQQKPGQPPRLLIYAASNLESGIPARFSGSGSGTDFTLTISSVEPEDFATYYCQQSNEDPPTFGGGTKVEIKRTVAAPSVFIFPPSDEQLKSGTASVVCLLNNFYPREAKVQWKVDNALQSGNSQESVTEQDSKDSTYSLSSTLTLSKADYEKHKVYACEVTHQGLSSPVTKSFNRGEC